European Patent Application EP 4 361 175 A1, published May 1, 2024. Title: Receptor-type tyrosine kinase agonist, cell culture medium composition, and undifferentiability maintenance composition. Applicant: Sekisui Chemical Co., Ltd. Epsilon Molecular Engineering, Inc. The sequence listing filed with the application follows.

SEQUENCE LISTING (58 sequences)

SEQ ID NO: 1 - DNA, 51 bp, Artificial Sequence
  primer
cattttacattctacaactacaagccaccatggctgagttgcagctcgtgg

SEQ ID NO: 2 - DNA, 70 bp, Artificial Sequence
  primer
gccgccgtgatgatgatgatgatggctaccacctcccgattgtggttttggtgtcttgggttctgaggag

SEQ ID NO: 3 - DNA, 60 bp, Artificial Sequence
  primer
gccgccgtgatgatgatgatgatggctaccacctcccgattgtggttttggtgtcttggg

SEQ ID NO: 4 - DNA, 117 bp, Artificial Sequence
  primer
gatcccgcgaaattaatacgactcactataggggaagtatttttacaacaattaccaacaacaacaacaaacaacaacaacattacattttacattctacaactacaagccaccatg

SEQ ID NO: 5 - DNA, 61 bp, Artificial Sequence
  primer
tttccacgccgccccccgtcctgcttccgccgtgatgatgatgatgatggctgcctccccc

SEQ ID NO: 6 - DNA, 22 bp, Artificial Sequence
  primer
tttccacgccgccccccgtcct

SEQ ID NO: 7 - DNA, 60 bp, Artificial Sequence
  primer
gatcccgcgaaattaatacgactcactataggggaagtatttttacaacaattaccaaca

SEQ ID NO: 8 - DNA, 58 bp, Artificial Sequence
  primer
  misc_feature (34)..(37): n is a, c, g, or t
tcgtcggcagcgtcagatgtgtataagagacagnnnnatggctgaggtgcagctcgtg

SEQ ID NO: 9 - DNA, 63 bp, Artificial Sequence
  primer
  misc_feature (35)..(38): n is a, c, g, or t
gtctcgtgggctcggagatgtgtataagagacagnnnntgatgatgatggctaccacctcccg

SEQ ID NO: 10 - DNA, 41 bp, Artificial Sequence
  primer
ccggccatggccactgcggccsagktgcagctcgtggagtc

SEQ ID NO: 11 - DNA, 44 bp, Artificial Sequence
  primer
gcctgcggccgcgtgatgatgatgatgatgggatcctccccccg

SEQ ID NO: 12 - protein, 5 aa, Artificial Sequence
  linker
GSGGG

SEQ ID NO: 13 - protein, 10 aa, Artificial Sequence
  lker
GSGGGGSGGG

SEQ ID NO: 14 - protein, 20 aa, Artificial Sequence
  linker
GSGGGGSGGGGSGGGGSGGG

SEQ ID NO: 15 - protein, 12 aa, Artificial Sequence
  linker
GSAGSAAGSGEF

SEQ ID NO: 16 - protein, 16 aa, Artificial Sequence
  linker
GSEGKSSGSGSESKST

SEQ ID NO: 17 - protein, 125 aa, Artificial Sequence
  VHH_Clone_#1
QLQLVESGGGSVQAGGSLRLSCAASRSLSRFNVWTWYRQAPVKQRELVASITKSGDTNYAESVKGRFIISRDDDKNTVYLQMNNLKSEDTGIYYCAGSYYSGSYLYPSPGGFSVWGQGTQVTVSS

SEQ ID NO: 18 - protein, 125 aa, Artificial Sequence
  VHH_Clone_#2
QVQLVESGGGLVQAGGSLRLSCAVPGSIFRFNTMGWYRQPPGKQRELVAQMSRGGITKYGDSVKGRFTITRDNAKNTVHLQMNSLKPEDTAVYYCAGSYYSGSYYYPSPQGFSVWGQGTQVTVSP

SEQ ID NO: 19 - protein, 255 aa, Artificial Sequence
  #1-5aa-#1
QLQLVESGGGSVQAGGSLRLSCAASRSLSRFNVWTWYRQAPVKQRELVASITKSGDTNYAESVKGRFIISRDDDKNTVYLQMNNLKSEDTGIYYCAGSYYSGSYLYPSPGGFSVWGQGTQVTVSSGSGGGQLQLVESGGGSVQAGGSLRLSCAASRSLSRFNVWTWYRQAPVKQRELVASITKSGDTNYAESVKGRFIISRDDDKNTVYLQMNNLKSEDTGIYYCAGSYYSGSYLYPSPGGFSVWGQGTQVTVSS

SEQ ID NO: 20 - protein, 260 aa, Artificial Sequence
  #1-10aa-#1
QLQLVESGGGSVQAGGSLRLSCAASRSLSRFNVWTWYRQAPVKQRELVASITKSGDTNYAESVKGRFIISRDDDKNTVYLQMNNLKSEDTGIYYCAGSYYSGSYLYPSPGGFSVWGQGTQVTVSSGSGGGGSGGGQLQLVESGGGSVQAGGSLRLSCAASRSLSRFNVWTWYRQAPVKQRELVASITKSGDTNYAESVKGRFIISRDDDKNTVYLQMNNLKSEDTGIYYCAGSYYSGSYLYPSPGGFSVWGQGTQVTVSS

SEQ ID NO: 21 - protein, 270 aa, Artificial Sequence
  #1-20aa-#1
QLQLVESGGGSVQAGGSLRLSCAASRSLSRFNVWTWYRQAPVKQRELVASITKSGDTNYAESVKGRFIISRDDDKNTVYLQMNNLKSEDTGIYYCAGSYYSGSYLYPSPGGFSVWGQGTQVTVSSGSGGGGSGGGGSGGGGSGGGQLQLVESGGGSVQAGGSLRLSCAASRSLSRFNVWTWYRQAPVKQRELVASITKSGDTNYAESVKGRFIISRDDDKNTVYLQMNNLKSEDTGIYYCAGSYYSGSYLYPSPGGFSVWGQGTQVTVSS

SEQ ID NO: 22 - protein, 262 aa, Artificial Sequence
  #1-L3-#1
QLQLVESGGGSVQAGGSLRLSCAASRSLSRFNVWTWYRQAPVKQRELVASITKSGDTNYAESVKGRFIISRDDDKNTVYLQMNNLKSEDTGIYYCAGSYYSGSYLYPSPGGFSVWGQGTQVTVSSGSAGSAAGSGEFQLQLVESGGGSVQAGGSLRLSCAASRSLSRFNVWTWYRQAPVKQRELVASITKSGDTNYAESVKGRFIISRDDDKNTVYLQMNNLKSEDTGIYYCAGSYYSGSYLYPSPGGFSVWGQGTQVTVSS

SEQ ID NO: 23 - protein, 266 aa, Artificial Sequence
  #1-L4-#1
QLQLVESGGGSVQAGGSLRLSCAASRSLSRFNVWTWYRQAPVKQRELVASITKSGDTNYAESVKGRFIISRDDDKNTVYLQMNNLKSEDTGIYYCAGSYYSGSYLYPSPGGFSVWGQGTQVTVSSGSEGKSSGSGSESKSTQLQLVESGGGSVQAGGSLRLSCAASRSLSRFNVWTWYRQAPVKQRELVASITKSGDTNYAESVKGRFIISRDDDKNTVYLQMNNLKSEDTGIYYCAGSYYSGSYLYPSPGGFSVWGQGTQVTVSS

SEQ ID NO: 24 - protein, 255 aa, Artificial Sequence
  #2-5aa-#2
QVQLVESGGGLVQAGGSLRLSCAVPGSIFRFNTMGWYRQPPGKQRELVAQMSRGGITKYGDSVKGRFTITRDNAKNTVHLQMNSLKPEDTAVYYCAGSYYSGSYYYPSPQGFSVWGQGTQVTVSPGSGGGQVQLVESGGGLVQAGGSLRLSCAVPGSIFRFNTMGWYRQPPGKQRELVAQMSRGGITKYGDSVKGRFTITRDNAKNTVHLQMNSLKPEDTAVYYCAGSYYSGSYYYPSPQGFSVWGQGTQVTVSP

SEQ ID NO: 25 - protein, 260 aa, Artificial Sequence
  #2-10aa-#2
QVQLVESGGGLVQAGGSLRLSCAVPGSIFRFNTMGWYRQPPGKQRELVAQMSRGGITKYGDSVKGRFTITRDNAKNTVHLQMNSLKPEDTAVYYCAGSYYSGSYYYPSPQGFSVWGQGTQVTVSPGSGGGGSGGGQVQLVESGGGLVQAGGSLRLSCAVPGSIFRFNTMGWYRQPPGKQRELVAQMSRGGITKYGDSVKGRFTITRDNAKNTVHLQMNSLKPEDTAVYYCAGSYYSGSYYYPSPQGFSVWGQGTQVTVSP

SEQ ID NO: 26 - protein, 270 aa, Artificial Sequence
  #2-20aa-#2
QVQLVESGGGLVQAGGSLRLSCAVPGSIFRFNTMGWYRQPPGKQRELVAQMSRGGITKYGDSVKGRFTITRDNAKNTVHLQMNSLKPEDTAVYYCAGSYYSGSYYYPSPQGFSVWGQGTQVTVSPGSGGGGSGGGGSGGGGSGGGQVQLVESGGGLVQAGGSLRLSCAVPGSIFRFNTMGWYRQPPGKQRELVAQMSRGGITKYGDSVKGRFTITRDNAKNTVHLQMNSLKPEDTAVYYCAGSYYSGSYYYPSPQGFSVWGQGTQVTVSP

SEQ ID NO: 27 - protein, 262 aa, Artificial Sequence
  #2-L3-#2
QVQLVESGGGLVQAGGSLRLSCAVPGSIFRFNTMGWYRQPPGKQRELVAQMSRGGITKYGDSVKGRFTITRDNAKNTVHLQMNSLKPEDTAVYYCAGSYYSGSYYYPSPQGFSVWGQGTQVTVSPGSAGSAAGSGEFQVQLVESGGGLVQAGGSLRLSCAVPGSIFRFNTMGWYRQPPGKQRELVAQMSRGGITKYGDSVKGRFTITRDNAKNTVHLQMNSLKPEDTAVYYCAGSYYSGSYYYPSPQGFSVWGQGTQVTVSP

SEQ ID NO: 28 - protein, 266 aa, Artificial Sequence
  #2-L4-#2
QVQLVESGGGLVQAGGSLRLSCAVPGSIFRFNTMGWYRQPPGKQRELVAQMSRGGITKYGDSVKGRFTITRDNAKNTVHLQMNSLKPEDTAVYYCAGSYYSGSYYYPSPQGFSVWGQGTQVTVSPGSEGKSSGSGSESKSTQVQLVESGGGLVQAGGSLRLSCAVPGSIFRFNTMGWYRQPPGKQRELVAQMSRGGITKYGDSVKGRFTITRDNAKNTVHLQMNSLKPEDTAVYYCAGSYYSGSYYYPSPQGFSVWGQGTQVTVSP

SEQ ID NO: 29 - protein, 17 aa, Artificial Sequence
  #1-CDR
SYYSGSYLYPSPGGFSV

SEQ ID NO: 30 - protein, 17 aa, Artificial Sequence
  #2-CDR
SYYSGSYYYPSPQGFSV

SEQ ID NO: 31 - protein, 25 aa, Artificial Sequence
  humanized VHH
QVQLVESGGGLVQPGGSLRLSCAAS

SEQ ID NO: 32 - protein, 17 aa, Artificial Sequence
  humanized VHH
LGWFRQAPGQGLEAVAA

SEQ ID NO: 33 - protein, 39 aa, Artificial Sequence
  humanized VHH
YYADSVKGRFTISRDNSKNTLYLQMNSLRAEDTAVYYCA

SEQ ID NO: 34 - protein, 11 aa, Artificial Sequence
  humanized VHH
WGQGTLVTVSS

SEQ ID NO: 35 - protein, 25 aa, Artificial Sequence
  human VH reference
QVQLVQSGGGLVQPGGSLRLSCAAS

SEQ ID NO: 36 - protein, 15 aa, Artificial Sequence
  human VH reference
WVRQAPGKGLEWVSP

SEQ ID NO: 37 - protein, 39 aa, Artificial Sequence
  human VH reference
YYADSVKGRFTISRDNSKNTLYLQMNTLRAEDTAVYYCA

SEQ ID NO: 38 - protein, 11 aa, Artificial Sequence
  human VH reference
WGQGTMVTVSS

SEQ ID NO: 39 - protein, 25 aa, Artificial Sequence
  universal VHH
QVQLVESGGGSVQPGGSLRLSCTAS

SEQ ID NO: 40 - protein, 17 aa, Artificial Sequence
  universal VHH
LGWFRQAPGQEREAVAA

SEQ ID NO: 41 - protein, 39 aa, Artificial Sequence
  universal VHH
YYADSVKGRFTISRDNAKNTVTLQMNNLKPEDTAIYYCA

SEQ ID NO: 42 - protein, 11 aa, Artificial Sequence
  universal VHH
WGQGTQVTVSS

SEQ ID NO: 43 - protein, 25 aa, Artificial Sequence
  CAMDR
EVQLVESGGGSVQAGGSLRLSCAAS

SEQ ID NO: 44 - protein, 14 aa, Artificial Sequence
  CAMDR
WYRQAPGKEREFVS

SEQ ID NO: 45 - protein, 39 aa, Artificial Sequence
  CAMDR
YADSVKGRFTISQDNAKNTVYLQMNSLIPEDTAMYYCKT

SEQ ID NO: 46 - protein, 11 aa, Artificial Sequence
  CAMDR
WGQGTMVTVSS

SEQ ID NO: 47 - protein, 25 aa, Artificial Sequence
  LAMGL
QVQLQESGGGLVQPGGSLRLSCTAS

SEQ ID NO: 48 - protein, 14 aa, Artificial Sequence
  LAMGL
WYRQAPGSKREFVA

SEQ ID NO: 49 - protein, 39 aa, Artificial Sequence
  LAMGL
FADSVKGRFTISRDNAKTTVDLQMNSLKPEDTAVYYCAA

SEQ ID NO: 50 - protein, 11 aa, Artificial Sequence
  LAMGL
WGKGTQVTVSS

SEQ ID NO: 51 - protein, 25 aa, Artificial Sequence
  VICPA
QVQLVETGGGLVQTGGSLRLSCKAS

SEQ ID NO: 52 - protein, 14 aa, Artificial Sequence
  VICPA
WFRQAPGKERDFVA

SEQ ID NO: 53 - protein, 40 aa, Artificial Sequence
  VICPA
TYADSVKGRFTISRDNASNMVYLLMNNLKPEDTAVYYCAA

SEQ ID NO: 54 - protein, 11 aa, Artificial Sequence
  VICPA
WGQGTQVTVSS

SEQ ID NO: 55 - DNA, 27 bp, Artificial Sequence
  linker
aagaatttccakgccgccccccgvcct

SEQ ID NO: 56 - DNA, 42 bp, Artificial Sequence
  rimer-F
ttgcacttgtcacgaattcgcagttgcagctcgtggagtctg

SEQ ID NO: 57 - DNA, 44 bp, Artificial Sequence
  Primer-R
tgtcagatctaaccatggccgatgaggagacggtgacctgggtc

SEQ ID NO: 58 - protein, 155 aa, Homo sapiens [sequence omitted]